European Patent Application EP 4 772 643 A1, published July 8, 2026. Title: A microorganism introduced with exogenous nicotinamide nucleotide transhydrogenase and method for producing L-amino acid or its derivative using the same. Applicant: 씨제이제일제당 주식회사. The sequence listing filed with the application follows.

SEQUENCE LISTING (50 sequences)

SEQ ID NO: 1 - DNA, 35 bp, synthetic construct
  source 1..35: mol_type = other DNA
aattcgagctcggtacccaatggagctgaaagaat

SEQ ID NO: 2 - DNA, 30 bp, synthetic construct
  source 1..30: mol_type = other DNA
cttcctgatagtcccgggacattgtttttc

SEQ ID NO: 3 - DNA, 30 bp, synthetic construct
  source 1..30: mol_type = other DNA
gaaaaacaatgtcccgggactatcaggaag

SEQ ID NO: 4 - DNA, 38 bp, synthetic construct
  source 1..38: mol_type = other DNA
gtcgactctagaggatccccataaaaacaggcagagga

SEQ ID NO: 5 - DNA, 35 bp, synthetic construct
  source 1..35: mol_type = other DNA
cctgaaaaacaatgtcccaacgaccgagcctattg

SEQ ID NO: 6 - DNA, 20 bp, synthetic construct
  source 1..20: mol_type = other DNA
gttgtgtctcctctaaagat

SEQ ID NO: 7 - DNA, 37 bp, synthetic construct
  source 1..37: mol_type = other DNA
tctttagaggagacacaacatgctgattggtattccc

SEQ ID NO: 8 - DNA, 36 bp, synthetic construct
  source 1..36: mol_type = other DNA
caacttcctgatagtcccttacagcgcggaggtgat

SEQ ID NO: 9 - DNA, 32 bp, synthetic construct
  source 1..32: mol_type = other DNA
agaggagacacaacatgcgaattggcatacca

SEQ ID NO: 10 - DNA, 35 bp, synthetic construct
  source 1..35: mol_type = other DNA
aacttcctgatagtcccttacagagctttcaggat

SEQ ID NO: 11 - DNA, 35 bp, synthetic construct
  source 1..35: mol_type = other DNA
tctttagaggagacacaacgtgcgtatcggtattc

SEQ ID NO: 12 - DNA, 38 bp, synthetic construct
  source 1..38: mol_type = other DNA
accaacttcctgatagtcccttagttgctgatccctgc

SEQ ID NO: 13 - DNA, 39 bp, synthetic construct
  source 1..39: mol_type = other DNA
atctttagaggagacacaacatgagaatcggcatccctt

SEQ ID NO: 14 - DNA, 34 bp, synthetic construct
  source 1..34: mol_type = other DNA
ccaacttcctgatagtcccttaagcgttgacctt

SEQ ID NO: 15 - DNA, 37 bp, synthetic construct
  source 1..37: mol_type = other DNA
atctttagaggagacacaacatgcgcatcggtgtgcc

SEQ ID NO: 16 - DNA, 32 bp, synthetic construct
  source 1..32: mol_type = other DNA
acttcctgatagtccctcaacccacccgcagc

SEQ ID NO: 17 - DNA, 39 bp, synthetic construct
  source 1..39: mol_type = other DNA
tctttagaggagacacaacatgcttattggtattccgag

SEQ ID NO: 18 - DNA, 41 bp, synthetic construct
  source 1..41: mol_type = other DNA
aaccaacttcctgatagtcccctacaggtgggagatgatct

SEQ ID NO: 19 - DNA, 472 bp, synthetic construct
  source 1..472: mol_type = other DNA
aacgaccgagcctattgggattaccattgaagccagtgtgagttgcatcacattggcttcaaatctgagactttaatttgtggattcacgggggtgtaatgtagttcataattaaccccattcgggggagcagatcgtagtgcgaacgatttcaggttcgttccctgcaaaaactatttagcgcaagtgttggaaatgcccccgtttggggtcaatgtccatttttgaatgtgtctgtatgattttgcatctgctgcgaaatctttgtttccccgctaaagttgaggacaggttgacacggagttgactcgacgaattatccaatgtgagtaggtttggtgcgtgagttggaaaaattcgccatactcgcccttgggttctgtcagctcaagaattcttgagtgaccgatgctctgattgacctaactgcttgacacattgcatttcctacaatctttagaggagacacaac

SEQ ID NO: 20 - protein, 513 aa, Corynebacterium variabile
MLIGIPREPQTLVAATPDTVGKLIKLGYDVAVQSGAGDQANHPDSQYESAGARIVGDDVWSTADIITTLDTPSAEQRAAMKPQATLIARLAPGRNDELVADLAAKNLTAMAMDTVPRISRAQAMDVLSSQANVAGYRAVIEAANTFGRLFTGQVTAAGKVPPATVYVIGTGVAGLAAIGTANSMGAVVKATDLRPETAEQVESMGAEFVAIPTASEKSDDGYAKEMTQDQAAAAAKLYAEQAARADIVITTANIPGRKSPVLLTAADVAAMTPGSVIVDMAAANGGNCELTVPGEVTETDNGVKIIGYTDLAGRLPAQSSQLYGQNIVNLFKLVTPGKDGRLVLDMDDEIVRGITVTQASATGSASDILWPPPPVKVSAAPAPAPAAATAAAEAEEEEPKGSGLWWKIVAGALGVALVLASPLSVTTNYMILMLAVVVGFYVITAVSHSLHTPLMSETNAISGIILVGAVLQVGSSNAAIAVLAFIAVVIASINIFGGFAVTRRMLAMFQGGN

SEQ ID NO: 21 - protein, 499 aa, Corynebacterium variabile
MNSFILATEVTNPDVSQDLLDWTDRISTLAYLVAALLFILALAGLSKQQSASRGNTFGIAGMTIALVATVFKAAVQSHADPENYNDAWVTILLVAVAMLIGAVIGIARASKVEMTGMPELIAMLHCFVGAAAVLIGVNSFIHAEHTSEAGYEKFHLGEVYLGIFIGAVTFTGSIIAYLKLSARMKGAPLTLPGRNLLNLAIIVLSVVGMVFFILTGTEEADNKAVAWTILGIMIVLALLLGLHLVAAIGGGDMPVVVSMLNSYSGWAAAAAGFMLANPLLIITGALVGSSGAYLSYIMCKAMNRSFISVILGGFGTEASSSDDRDYGTHTEITAEETAELLKGAKSVMITPGYGMAVAQAQYPVAAMVSKLREKGVDVTFGIHPVAGRLPGHMNVLLAEAKVPYDIVHEMDEVNDDFADIDVVLVIGANDTVNPIAEEPGSPLAGMPVLKVWEAKRVVVFKRSMGAGYAGVQNPLFFNENTDMLLGDAKDSVEKITSAL

SEQ ID NO: 22 - protein, 510 aa, Escherichia coli
MRIGIPRERLTNETRVAATPKTVEQLLKLGFTVAVESGAGQLASFDDKAFVQAGAEIVEGNSVWQSEIILKVNAPLDDEIALLNPGTTLVSFIWPAQNPELMQKLAERNVTVMAMDSVPRISRAQSLDALSSMANIAGYRAIVEAAHEFGRFFTGQITAAGKVPPAKVMVIGAGVAGLAAIGAANSLGAIVRAFDTRPEVKEQVQSMGAEFLELDFKEEAGSGDGYAKVMSDAFIKAEMELFAAQAKEVDIIVTTALIPGKPAPKLITREMVDSMKAGSVIVDLAAQNGGNCEYTVPGEIFTTENGVKVIGYTDLPGRLPTQSSQLYGTNLVNLLKLLCKEKDGNITVDFDDVVIRGVTVIRAGEITWPAPPIQVSAQPQAAQKAAPEVKTEEKCTCSPWRKYALMALAIILFGWMASVAPKEFLGHFTVFALACVVGYYVVWNVSHALHTPLMSVTNAISGIIVVGALLQIGQGGWVSFLSFIAVLIASINIFGGFTVTQRMLKMFRKN

SEQ ID NO: 23 - protein, 462 aa, Escherichia coli
MSGGLVTAAYIVAAILFIFSLAGLSKHETSRQGNNFGIAGMAIALIATIFGPDTGNVGWILLAMVIGGAIGIRLAKKVEMTEMPELVAILHSFVGLAAVLVGFNSYLHHDAGMAPILVNIHLTEVFLGIFIGAVTFTGSVVAFGKLCGKISSKPLMLPNRHKMNLAALVVSFLLLIVFVRTDSVGLQVLALLIMTAIALVFGWHLVASIGGADMPVVVSMLNSYSGWAAAAAGFMLSNDLLIVTGALVGSSGAILSYIMCKAMNRSFISVIAGGFGTDGSSTGDDQEVGEHREITAEETAELLKNSHSVIITPGYGMAVAQAQYPVAEITEKLRARGINVRFGIHPVAGRLPGHMNVLLAEAKVPYDIVLEMDEINDDFADTDTVLVIGANDTVNPAAQDDPKSPIAGMPVLEVWKAQNVIVFKRSMNTGYAGVQNPLFFKENTHMLFGDAKASVDAILKAL

SEQ ID NO: 24 - protein, 517 aa, Corynebacterium urealyticum
MRIGIPVEPGENQPLVAATPDTVGKLIKLGYDVEVQAGAGEDAAYPDALYREAGASIVGEEVWEADIVTTLDTPPKEKRDLMRSGATLICRMAPGRNEELINELANRGITGLAMDAVPRISRAQSMDVLSSMANIAGYRAVIEAANAFGRLFTGQVTAAGKVPPAKVYVIGAGVAGLAAIGTANSMGAIVKATDLRVEAGEQVESMGAEFVAIQEEAEKSEDGYAKEMTQDQAELAAKIYSQQSAEADIVITTANIPGRTSPVLLTEEDVANMRPGSVVVDLAAANGGNCALTKPGEVFVTDNGVTIIGYTDLAGRLPGQASQLFGQNIVNLFKLITPEKDGQRVLDLDDEIIRTITVTLNDGQETSVLWPPPPVSVSVAPQQQPAQDTQAAEEPEKQAFMGGPFAKIGLAIAILLGAAIVLVSPLGMSGNFVVLTLAIVLGFYVISAVTPTLHTPLMSETNAISGIVLVGAILQVNSPNIIVTVLAFLAIVVSSVNVFGGFAITDRMLGMFVKEDA

SEQ ID NO: 25 - protein, 495 aa, Corynebacterium urealyticum
MTATLILSQAATGENATLLDWLARISNLAYIVAAVLFLMALAGLSKPETAKRGNTLGMSGMAVAIAVAIFQAVVHSTTDSDALDPVITVVLIALAMSLGAAYGIKRAHSVEMTGLPQLIALFNGMVGLGAVFIGYNSFVSESADSMGAAAYNFHLGEVFLGIFIGAVTFTGSILAGLKLSGKVKGAPLLLPARNLLNVAILVISLVLMVVFILAGEGTTAWIAVGIMTALALFMGWHLVAAIGGGDMPVVVSIMNSYSGWAAAFTGLMLQNPLLIITGALVGSSGAFLSYVMCQAMNRSFLNVLLGGFGTDGGAVAEGVDGTHTEIDTDEAVAMLKDAKNIMITPGYGMAVSQAQYTVAELTRKLRDQGKTVQFGIHPVAGRLPGHMNVLLAEAKVPYDIVMDMEEINDDFDEVDVVLVIGANDTVNPSAEMPGSPIAGMPVLKVWEAERVIVLKRSMGAGYSGAQNPLFFNENTDMLLGDAKASIEKLAAGISN

SEQ ID NO: 26 - protein, 524 aa, Corynebacterium amycolatum
MRIGIPLEPDPQQTIVAATPETVGKLVKLGYDVAVQADAGLAAKFTDADYESAGAAIVDESVWHSDIVVTLDTPPEQFRALLNDGAMLVSRLAPGRNEELVEELAHRNITALAMDAVPRISRAQSMDVLSSMANIGGYRAVVEAASAYGRLFTGQVTAAGKMPPATVYVIGAGVGGLAAIGTANSMGAIVKATDLRPEAGEQVESMGAEFIPIPAATEKSEDGYAKEMTNDQAAAAAKLYSEQSAQADIVITTANIPGRRSPLLLTAADVAAMKPGSVIVDMAAAGGGNCEMTVPGKTIVTDNGVTIIGYTDLAGRLPAQASSLYGQNIFNLFKLITPEKDGSPVLNLEDEIIRGITVTKARPQNGAGATGAEILWPPPPIKVAVTPAAPLQEQQAQQAALEENAPEKVSFMGSGMGSKIALGLTALLAIVVMLSAPHSVSANFMVLTLAIVLGFYVISAVTPRLHTPLMSETNAISGIVLVGAILQVGSSNLLVSGLAFAAIVVSSINIFGGFAVTDRMLGMF

SEQ ID NO: 27 - protein, 491 aa, Corynebacterium amycolatum
MASIDTASLLDWTYRLSNVGYIVAAVLFLAALSGLSKPETARRGNAFGIAGMAVAVVIAIFQALVTADTKPDSHFSPLITLILIAVAIGIGGVIGISRARSVAMTGMPQLIALFNGLVGLGAIFIGFNSYIFAEDVAPDALKFHFGEVYIGVFIGAVTFTGSIVAGLKLSEKIKGSPLLLPGRNALNIAILVVTLVLLAVFIATGTEGGAIAWACMVAVTALGLFLGWHLVIAIGGGDMPVVVSIMNSYSGWAAAFTGLMLGNPLLIITGALVGSSGAYLSYIMCEAMNRSFANVILGGFGSEASSGSAVEGSHTEVSHEDTSEILRDADKILIAPGYGMAVAQAQYAVADLVRNLRDAGKEVVFGIHPVAGRLPGHMNVLLAEAKVPYDIVLELDEVNDDFADVDVTLVIGANDTVNPMAEQPGSPIAGMPVLKVWESERVIVLKRSMGSGYSGVQNPLFFNENTDMLIGDAKASIDSLNRILADSKVNA

SEQ ID NO: 28 - protein, 535 aa, Cellulosimicrobium funkei
MRIGVPREVRDGERLVAATPRTVERLRALGYDVVVEHDAGAGATFSDAAYEAAGAAVVDAAAAWGADVVTAVNAPTDAQVALLRPGATLVAMLGPANDPDLVQRLAAHGVTALALDAVPRISRAQALDVLSTLSNVAGYRAVVEAAGEYGGMFAGQVTAAGKTPPARVFVIGGGVAGLAAVGAAASLGAQVRAFDVRSEAAEQIESMGGTAVREPAAQQGMSADGYAKPLTPEQEAAALAVYAREAAEADVVITTALVRGRAPRTLTAEAVAGMRPGSVVVDLAASGGGNCALTVPGERVVTEDGVVVVGWTDLAGRLPQHTSQLLGTNVVHLLELLTPGKDGTLALDLDDPVQRGMTVARDGDVLWPPPPVAVSAAPAPGSTVPPPPPDPAQEAADRERAAAEAASAASLRRRRRTVGAALAAVLVTLALSFAPPSLVGHVTVFTLAVVVGYYVISNVTHSLHTPLMAQTNAISGIILVGALLQIGSDDWVVTTLALLAATVASINIFGGFLVANRMIRMFRKDAPARAQGVAR

SEQ ID NO: 29 - protein, 470 aa, Cellulosimicrobium funkei
MTATSVAQAVYVLAAVLFVLSLAGLSKQESARRGNLLGMVGMVLALAATIVLALGTSARPVLVTALLIALVLLVGAAVGTWRARRVEMTQMPELIAILHSFVGAAAVLVGFNSYLTAHAAGADDVAHLVEVSLGVLVGAVTFTGSVVAFLKLSGRTRSAPLQLPGRNLLNLAALLVSLGLVVWFVVAPSIWPLLLLTVVSLALGWHLVASIGGGDMPVVVSMLNSYSGWAAAAAGFMLGNDLLIVTGALVGSSGAILSYIMCKAMNRSFVSVILGGFGAEEGAAPAGGGEGPQGEHREVSADEVAALLRDARSVVITPGYGMAVAKAQYPVAELVELLRDGGAEVRFGVHPVAGRLPGHMNVLLAEARVPYDIVLEMDEINDDLAGTDVVLVIGANDTVNPAALDDPGSPIAGMPVLHVWEAGQVVVFKRSMAAGYAGVQNPLFFRENTGMLFGDAKQRVEDIVAALRVG

SEQ ID NO: 30 - protein, 514 aa, Corynebacterium zhongnanshanii
MLIGIPREPASLVSATPDTVGKLIKLGYDVAVQSGAGDDSNYPDSQYEEAGARIVGDEVWQSDIITALDEPTAEQRADLKPGAALIARLAPARNEQLIQEFADKNVTSIAMDTVPRISRAQSMDVLSSQANIAGYRAVIEAANTFGRLFTGQVTAAGKVPPAIVYVIGAGVAGLAAIGTANSMGAIVKATDLRPETAEQVESMGAEFVAIQAETEKSEDGYAKEMTADQAQAAAKLYAEQSAAADIVITTANIPGRKSPVLLTAADVAAMKPGSVIVDMAAANGGNCELTVPGEITVTDNGVSIIGYTDLAGRLPAQASQLYGQNIVNLLKLMTPGKDGQLVFDLEDEIVRGITVTHSTGEAAGSADILWPPPPVKVSAAPAQPAPAAAAAAGDQAEEAPAKKSGAWKVIAALLGIALILASPMQVAAEYMLLMLAIVVGFYVITAVTHKLHTPLMSETNAISGIILVGAILQVGSSNIAVAALSFVAIVVASINIFGGFFVTRRMLTMFDGGN

SEQ ID NO: 31 - protein, 495 aa, Corynebacterium zhongnanshanii
MNAFYFAQAEATSKVSPTVLEWTDKITNLAYIVAALLFILALAGLAKQQTASRGNRFGMAGMTIALIATIAKAVINAKDGGDATNGPIVTVLLIAVAMLLGAAIGIPRAKKVEMTEMPELIAMLHSFVGLAAVLIGVNSFIQPDEKTKAIEAFHLGEVYLGVFIGAVTLTGSIVAYLKLSGKMNGKPLVLPARHLLNLLVIIVSLVGMVVFIASGHDNQVLSWIALVVMLALALFLGFHLVAAIGGGDMPVVVSMLNSYSGWAAAAAGFMLGNPLLIIVGALVGSSGAYLSYVMCQAMNRSFVSVILGGFGGEAAASDDREYGEHTEVNAAETAELLKGAKTVMITPGYGMAVAQAQYPVATLVEKLKAQGVDVTFGIHPVAGRLPGHMNVLLAEAKVPYDIVLELDEVNDDFADIDVVLVIGANDTVNPIAEEPGSPIAGMPVLKVWEADKVIVFKRSMGSGYAGVQNPLFFNENTDMLLGDAKKTVEEIISHL

SEQ ID NO: 32 - DNA, 18 bp, synthetic construct
  source 1..18: mol_type = other DNA
cgacatcgaacagcgttc

SEQ ID NO: 33 - DNA, 18 bp, synthetic construct
  source 1..18: mol_type = other DNA
cattggataattcgtcga

SEQ ID NO: 34 - DNA, 18 bp, synthetic construct
  source 1..18: mol_type = other DNA
ctcttccgatgaccgtga

SEQ ID NO: 35 - DNA, 18 bp, synthetic construct
  source 1..18: mol_type = other DNA
cttaggtatcatgggtgg

SEQ ID NO: 36 - DNA, 18 bp, synthetic construct
  source 1..18: mol_type = other DNA
tgtgccaggccatgaacc

SEQ ID NO: 37 - DNA, 18 bp, synthetic construct
  source 1..18: mol_type = other DNA
cttaggtatcatgggtgg

SEQ ID NO: 38 - DNA, 1542 bp, Corynebacterium variabile
  source 1..1542: mol_type = other DNA
atgctgattggtattccccgtgaaccccagacccttgttgctgcgaccccggacaccgttggtaaactgattaaactcggctatgacgttgcagtgcagtccggcgccggtgatcaagctaaccacccagactcccagtacgaatctgctggcgcgcgcattgtgggtgatgacgtctggtccaccgcagacatcattaccaccctggacaccccttccgcagaacagcgtgcagccatgaagccacaagccaccttgatcgctcgccttgcgcctggccgtaacgatgagctggtggcagacctcgctgcgaaaaatctgaccgcaatggcaatggataccgttccgcgcatttcccgtgctcaggcgatggacgtgctctcctctcaagcaaacgttgcaggctaccgcgcagtgatcgaggcagcaaataccttcggccgtctgtttaccggtcaggtcaccgctgcgggtaaggttccacctgctaccgtctatgttattggcaccggtgtggcaggcttggcagccatcggcaccgcaaactctatgggcgcggtggtcaaagcaaccgatcttcgcccggaaaccgcagagcaggtggaatctatgggcgcagagttcgtcgctatccctaccgcgtccgaaaagtctgatgacggttacgccaaagagatgacccaggatcaagctgcggcagccgctaagctgtatgcagaacaggcggcacgcgccgacatcgtgattaccaccgcaaacattcctggccgtaaatccccggttctgctcaccgccgctgatgtggcggcaatgaccccaggttctgtgatcgtggatatggccgctgcgaacggcggtaattgcgaactgaccgttcctggcgaggtgaccgaaaccgataacggcgtgaagatcattggttacaccgacttggctggccgccttcctgcacagtcctctcaattgtatggtcagaacatcgtgaatctgttcaagctcgtcacccccggcaaagatggtcgcttggtccttgacatggatgacgaaattgtgcgtggcatcaccgtcacccaagcatccgccaccggttccgcttctgacatcctgtggccgcccccacctgttaaggtgtccgcagcccctgctcctgcaccagctgcggcaaccgccgctgcggaggcagaagaggaagagccaaagggctccggtctgtggtggaaaatcgtcgcaggcgccctcggtgtcgcactggttctcgcctcccctctctctgttaccaccaactacatgattttgatgcttgctgttgtggtcggcttttatgtcatcaccgcggttacccactccctgcacaccccactcatgtccgaaaccaatgctatttctggcatcattttggtgggtgcggtccttcaggttggctcctctaacgcagccatcgctgtcttggcgttcatcgcaattgttatcgcatccattaatatcttcggcggttttgctgtgacccgccgtatgcttgcgatgttccagggaggtaactga

SEQ ID NO: 39 - DNA, 1500 bp, Corynebacterium variabile
  source 1..1500: mol_type = other DNA
atgaactcttttattctggcgaccgaagtgaccaaccccgatgtgtctcaggatttgctggactggaccgaccgtatttctaccctcgcttaccttgtggcagccctgctcttcatcctcgctttggcgggtctgtctaagcagcaatccgctgcgcgcggcaacaccttcggtatcgctggtatgaccattgcgctcgttgcaaccgtgtttaaagcagccgtgcagtcccacgcagatccagagaactataatgacgcatgggtcaccatcttgcttgtcgcagttgccatgctgattggtgcagtcatcggcattgctcgcgcgtccaaggttgagatgaccggtatgccagaactcatcgccatgttgcactgcttcgtgggtgctgcggcagtgctgatcggcgtcaactcttttattcacgcggaacacacctccgaggcaggttacgaaaaattccaccttggcgaagtgtatctgggtatcttcattggcgcagtcacctttaccggctctatcattgcctaccttaagctgtccgcccgcatgaaaggtgctccgctcaccttgcccggccgtaacctgctcaatctcgcaatcattgtgttgtccgtggtcggtatggtcttctttatcctgaccggcaccgaagaggcagataacaaggcagttgcctggaccattcttggtatcatgattgtgctggccttgcttctgggtcttcacctggtcgcagctatcggtggtggtgacatgccggttgtggtctccatgctcaactcttactccggttgggcggcagccgctgcgggcttcatgttggctaatcccctcttgatcattaccggcgccctcgtcggttcctctggtgcttacttgtcctatatcatgtgtaaggctatgaaccgctctttcatctccgttattctgggtggctttggcaccgaagcgtcctcttccgatgaccgtgattatggcacccacaccgaggtcaccgcggaagagaccgcagaacttctgaagaacgccaaatccgttatgatcacccctggttacggtatggctgtggcacaggcacaatatcccgttgcagcaatggtgtccaagctgcgcgagaagggtgtggacgtcaccttcggcatccacccagtcgcaggtcgtctccctggccacatgaacgttctcttggccgaagctaaggtcccgtacgatattgttcacgaaatggacgaagtgaatgatgactttgccgacatcgacgttgtgctcgttattggcgccaacgataccgtgaatccaatcgctgaagagccaggttctcctattgcgggtatgccagtcttgaaggtttgggacgcaaaccgcgtcgttgtgttcaaacgctctatgggcgccggctacgctggcgttcaaaacccattgttctttaacgagaacaccgatatgcttctgggcgatgctaaggactctgtggaaaaaatcacctccgcgctgtaa

SEQ ID NO: 40 - DNA, 1545 bp, Corynebacterium zhongnanshanii
  source 1..1545: mol_type = other DNA
atgcttattggtattccgagagaaccagcctccctggtttcggccaccccagacaccgtaggcaagctcattaagcttggttacgacgttgccgttcaatctggagcgggcgacgattccaactaccccgactctcagtacgaagaagccggcgcgcgtatcgtcggcgatgaagtgtggcagtcggacatcatcaccgctctcgacgagcccaccgcagagcagcgagcagacctgaagccaggcgcggccctcatcgcccgtcttgcccctgcgcgcaacgagcagctgatccaggagttcgcagacaagaacgtcacctccatcgccatggacaccgtgccgcgtatcagccgtgcgcagtcgatggacgtgctgagctcccaggcgaacatcgccggctaccgcgccgtgattgaggctgccaacaccttcggccgcctgttcaccggtcaggtgaccgcagccggtaaggtgccgccagcgatcgtctacgtgattggtgcgggtgtggccggactggccgccatcggtaccgccaactccatgggtgcgatcgtcaaggcgacggacttgcgtccggagaccgccgagcaggtggaatccatgggtgcggagttcgttgccatccaggccgagaccgaaaagtctgaggacggctacgccaaggagatgaccgcggaccaagcccaggctgccgccaagctctacgctgagcagtccgccgccgcagacatcgtcatcaccaccgcgaacatccccggccgcaagtcccccgtgctgctgaccgcagccgacgttgccgccatgaagcccggctccgtcatcgtcgatatggccgcggccaacggcggtaactgtgagctgaccgtgccgggagagatcaccgtcaccgataacggtgtgagcatcatcggctacacggaccttgccggacgtctgcctgcacaggcatcccagctgtacggtcagaacatcgtgaacttgctgaagctcatgaccccaggcaaggacggccagctggtcttcgacctggaggacgagatcgttcgcggtatcaccgtcacgcactccaccggggaggcagccggatcggccgacatcctgtggccgccaccaccagtgaaggtctccgctgcgcctgcgcagccagcacccgcagctgctgctgccgctggcgaccaggccgaggaggcccctgccaagaagtccggcgcgtggaaggtcatcgccgcactgctgggtatcgctctgatcttggccagcccgatgcaggttgctgcagagtacatgctgctgatgctcgcgatcgtggtgggcttctacgtgatcactgcggtgacgcataagctgcacaccccgctgatgagtgagaccaacgccatctccggcatcatccttgttggcgcaatcctgcaggtcggtagctcgaatatcgcggttgctgccctaagtttcgtggcgattgttgtggcctctatcaacattttcggtggcttcttcgtcacccgccgcatgctcaccatgttcgacggaggtaactaa

SEQ ID NO: 41 - DNA, 1488 bp, Corynebacterium zhongnanshanii
  source 1..1488: mol_type = other DNA
atgaacgctttttatttcgcacaggctgaggccacctctaaggtgagccccaccgtcctggaatggacggataagattacgaacctcgcgtatatcgttgcagcgctgctgttcatcctggccctggctggtttggccaagcagcagaccgcatcccgcggtaatcgcttcggcatggcgggtatgaccatcgcgctcatcgcgacgatcgccaaggctgtcattaacgcgaaggatgggggcgacgccaccaacggcccaattgtcaccgttttgctgatcgctgtggcgatgctgctgggtgccgcgattggtatcccacgggcgaagaaggtcgaaatgaccgaaatgccggaactcattgcgatgctgcacagcttcgtgggtcttgcggcagtgctgattggtgtgaactccttcatccagcccgatgagaagaccaaggccatcgaggccttccacctgggtgaggtctacctgggcgtgttcatcggtgctgtgaccctgaccggttccatcgtggcgtacctgaagctgagcggaaagatgaacggtaagccactggtgcttcctgctcgtcacttgctgaacctgctggtaatcatcgtgtccctggtgggcatggttgtgttcatcgcgtccggtcacgacaatcaggtcctgtcctggatcgcgctggtcgtgatgctggccctggctctgttcctgggattccacctggttgccgccatcggtggtggcgacatgccagtggttgtgtccatgctgaactcctactccggttgggcagctgctgccgctggattcatgctgggtaaccctctgctcatcatcgttggtgcgctggttggttcctccggtgcatacctgtcctacgtcatgtgccaggccatgaaccgtagcttcgtgtccgtgatcctgggtggcttcggtggcgaggctgctgcttctgacgaccgcgagtacggtgagcacaccgaggttaacgcggctgagaccgcggagctgctgaagggtgcgaagaccgtcatgatcaccccgggctacggcatggctgtggcgcaggctcagtacccagtggccaccctggtagagaagctcaaggctcagggcgtggatgttacgttcggtattcaccctgttgctggccgcctgcctggccacatgaacgtgctgctggccgaggctaaggtgccgtacgacatcgtgctggagctggatgaggtcaacgacgacttcgccgacatcgacgttgtgctggtcatcggtgcaaacgacacggtgaacccgatcgccgaagagcctggctcgccaattgccggcatgcctgtgctgaaggtgtgggaagcagacaaggtcatcgtctttaagcgttccatgggctccggttacgctggcgtgcagaacccactgttcttcaacgagaacacggacatgctgctcggcgatgcaaagaagaccgtggaggagatcatctcccacctgtag

SEQ ID NO: 42 - DNA, 1533 bp, Escherichia coli
  source 1..1533: mol_type = other DNA
atgcgaattggcataccaagagaacggttaaccaatgaaacccgtgttgcagcaacgccaaaaacagtggaacagctgctgaaactgggttttaccgtcgcggtagagagcggcgcgggtcaactggcaagttttgacgataaagcgtttgtgcaagcgggcgctgaaattgtagaagggaatagcgtctggcagtcagagatcattctgaaggtcaatgcgccgttagatgatgaaattgcgttactgaatcctgggacaacgctggtgagttttatctggcctgcgcagaatccggaattaatgcaaaaacttgcggaacgtaacgtgaccgtgatggcgatggactctgtgccgcgtatctcacgcgcacaatcgctggacgcactaagctcgatggcgaacatcgccggttatcgcgccattgttgaagcggcacatgaatttgggcgcttctttaccgggcaaattactgcggccgggaaagtgccaccggcaaaagtgatggtgattggtgcgggtgttgcaggtctggccgccattggcgcagcaaacagtctcggcgcgattgtgcgtgcattcgacacccgcccggaagtgaaagaacaagttcaaagtatgggcgcggaattcctcgagctggattttaaagaggaagctggcagcggcgatggctatgccaaagtgatgtcggacgcgttcatcaaagcggaaatggaactctttgccgcccaggcaaaagaggtcgatatcattgtcaccaccgcgcttattccaggcaaaccagcgccgaagctaattacccgtgaaatggttgactccatgaaggcgggcagtgtgattgtcgacctggcagcccaaaacggcggcaactgtgaatacaccgtgccgggtgaaatcttcactacggaaaatggtgtcaaagtgattggttataccgatcttccgggccgtctgccgacgcaatcctcacagctttacggcacaaacctcgttaatctgctgaaactgttgtgcaaagagaaagacggcaatatcactgttgattttgatgatgtggtgattcgcggcgtgaccgtgatccgtgcgggcgaaattacctggccggcaccgccgattcaggtatcagctcagccgcaggcggcacaaaaagcggcaccggaagtgaaaactgaggaaaaatgtacctgctcaccgtggcgtaaatacgcgttgatggcgctggcaatcattctttttggctggatggcaagcgttgcgccgaaagaattccttgggcacttcaccgttttcgcgctggcctgcgttgtcggttattacgtggtgtggaatgtatcgcacgcgctgcatacaccgttgatgtcggtcaccaacgcgatttcagggattattgttgtcggagcactgttgcagattggccagggcggctgggttagcttccttagttttatcgcggtgcttatagccagcattaatattttcggtggcttcaccgtgactcagcgcatgctgaaaatgttccgcaaaaattaa

SEQ ID NO: 43 - DNA, 1389 bp, Escherichia coli
  source 1..1389: mol_type = other DNA
atgtctggaggattagttacagctgcatacattgttgccgcgatcctgtttatcttcagtctggccggtctttcgaaacatgaaacgtctcgccagggtaacaacttcggtatcgccgggatggcgattgcgttaatcgcaaccatttttggaccggatacgggtaatgttggctggatcttgctggcgatggtcattggtggggcaattggtatccgtctggcgaagaaagttgaaatgaccgaaatgccagaactggtggcgatcctgcatagcttcgtgggtctggcggcagtgctggttggctttaacagctatctgcatcatgacgcgggaatggcaccgattctggtcaatattcacctgacggaagtgttcctcggtatcttcatcggggcggtaacgttcacgggttcggtggtggcgttcggcaaactgtgtggcaagatttcgtctaaaccattgatgctgccaaaccgtcacaaaatgaacctggcggctctggtcgtttccttcctgctgctgattgtatttgttcgcacggacagcgtcggcctgcaagtgctggcattgctgataatgaccgcaattgcgctggtattcggctggcatttagtcgcctccatcggtggtgcagatatgccagtggtggtgtcgatgctgaactcgtactccggctgggcggctgcggctgcgggctttatgctcagcaacgacctgctgattgtgaccggtgcgctggtcggttcttcgggggctatcctttcttacattatgtgtaaggcgatgaaccgttcctttatcagcgttattgcgggtggtttcggcaccgacggctcttctactggcgatgatcaggaagtgggtgagcaccgcgaaatcaccgcagaagagacagcggaactgctgaaaaactcccattcagtgatcattactccggggtacggcatggcagtcgcgcaggcgcaatatcctgtcgctgaaattactgagaaattgcgcgctcgtggtattaatgtgcgtttcggtatccacccggtcgcggggcgtttgcctggacatatgaacgtattgctggctgaagcaaaagtaccgtatgacatcgtgctggaaatggacgagatcaatgatgactttgctgataccgataccgtactggtgattggtgctaacgatacggttaacccggcggcgcaggatgatccgaagagtccgattgctggtatgcctgtgctggaagtgtggaaagcgcagaacgtgattgtctttaaacgttcgatgaacactggctatgctggtgtgcaaaacccgctgttcttcaaggaaaacacccacatgctgtttggtgacgccaaagccagcgtggatgcaatcctgaaagctctgtaa

SEQ ID NO: 44 - DNA, 1554 bp, Corynebacterium urealyticum
  source 1..1554: mol_type = other DNA
gtgcgtatcggtattccggttgagccgggtgagaaccagccgctggtggcagccacaccagacacggtcggcaagctcatcaagcttggctatgacgttgaagtacaggcaggtgccggcgaagacgccgcctaccctgacgccctctaccgcgaggccggcgcgagcatcgtaggcgaggaggtctgggaagcggacatcgtcacgacgctcgacaccccgcccaaggagaagcgcgacctcatgcgctccggagccaccctgatctgccgcatggctccaggccgcaacgaggagctcatcaacgagctcgccaaccgtggcatcaccgggctcgcgatggacgctgtgccgcgtatttcccgcgcacagtccatggatgtcctctcctccatggcaaacatcgccggctaccgcgcagtcatcgaggccgccaacgccttcggtcgactgttcaccggccaggtcaccgcggcaggtaaggtgccgccggcaaaggtctacgtcatcggcgctggtgtcgctggcctggccgcgatcggtaccgccaactccatgggcgcgatcgtcaaggccaccgacctgcgcgtcgaggcaggcgagcaggtcgagtccatgggggcggaattcgtcgccatccaggaagaggccgagaagtccgaggacggctacgccaaggagatgacccaagaccaggcggaactcgctgcgaagatctattcccagcagtccgccgaagccgacatcgtcatcaccaccgcaaacattccgggccgcacctcgccggtgctgctcaccgaggaagatgtcgccaacatgcgtccgggcagcgtcgtcgtcgacctggcggcagccaacggtggtaactgcgcgctgacgaagccgggcgaggtcttcgtcaccgataacggcgtgaccatcattggctacaccgacctggcgggccgcctgcctggccaggcctcccagctgttcggccagaacatcgtcaacctgttcaagctgatcacgccggagaaggacggccagcgcgtgctggacctggatgacgagatcatccgcaccatcaccgtcaccctcaatgacggccaggagacctccgtcctctggccgccaccaccggtgagcgtgtccgtcgccccgcagcagcagcccgcgcaggacacgcaggccgccgaggagccggagaagcaagccttcatgggtggccccttcgccaagatcggtctggccatcgccatcctactgggcgctgcaatcgtcctggtcagcccgctgggaatgagcggcaacttcgtcgtcctgaccctggccatcgtgctgggcttctacgtgatctccgctgtcaccccgaccctgcacaccccgttgatgtccgagacgaacgcgatttcaggaatcgtcctggtcggcgcgatcttgcaggtcaacagccccaatatcatcgttacggtcctcgcgttcctggcaatcgtcgtgtcctccgtcaacgtgttcggtggcttcgccatcacagaccgcatgctcggcatgttcgttaaggaggatgcataa

SEQ ID NO: 45 - DNA, 1488 bp, Corynebacterium urealyticum
  source 1..1488: mol_type = other DNA
atgactgccactctgattctttcgcaggcagcgaccggcgagaacgccacgctgctggattggctggcccggatctcgaacctggcctacatcgtggctgccgtgctcttcctcatggcactggccggcctctctaagccggagaccgcaaagcgcggtaacacgctgggcatgagcggtatggctgttgccatcgccgtggccatcttccaggccgtggttcactccaccaccgattccgatgccctggacccggtcatcaccgtcgtcctcattgccctggctatgagcctcggtgcggcctacggcatcaagcgcgcgcactccgtcgagatgactggtctgccgcagctgatcgcgctgttcaacggcatggtcggtctgggcgcggtcttcatcggctacaactccttcgtttccgagtccgccgactcgatgggtgctgccgcctacaacttccacctgggtgaggtcttcctcggcatcttcatcggtgccgtgaccttcaccggctcgatcctggctggcctgaagctctccggcaaggtcaagggcgccccgctgctgctgccggcccgtaacctgctgaacgtcgccatcctggtgatcagcctcgtgctcatggtcgtgttcatcctcgcgggtgaaggcaccaccgcctggatcgcggttggcatcatgaccgccctggcgctgttcatgggctggcacctggtcgctgccattggcggtggcgacatgccggtcgtcgtgtccatcatgaactcctactccggctgggcagctgccttcaccggtctgatgctgcagaacccgctgctgatcatcaccggtgcgctggtcggttcctccggtgcattcctctcctacgtgatgtgccaggcgatgaaccgctccttcctgaacgtcctgctgggcggcttcggcaccgacggtggcgcggtcgcggagggtgtcgacggcacccacaccgagatcgacaccgacgaggctgtcgcgatgctcaaggacgcgaagaacatcatgatcaccccgggctacggcatggctgtctcccaagcgcagtacacggtcgctgagctgacccgcaagctgcgcgaccagggtaagactgtccagttcggtatccacccggtcgccggtcgcctgcctggccacatgaacgtcctgctggctgaggcgaaggtcccttatgacatcgtcatggatatggaggagatcaacgacgacttcgacgaggtcgacgtggtcctggtcatcggcgcgaacgatacggtcaacccgagcgctgagatgccgggctccccgatcgccggcatgccggttctgaaggtgtgggaggctgagcgcgtgatcgtgctgaagcgttccatgggtgccggttactccggtgcgcagaacccgctgttcttcaacgagaacaccgacatgctgctcggtgatgcgaaggcatccatcgagaagctggccgcagggatcagcaactaa

SEQ ID NO: 46 - DNA, 1590 bp, Corynebacterium amycolatum
  source 1..1590: mol_type = other DNA
atgagaatcggcatccctttagaacccgatccccagcaaacaattgtggctgcgaccccggagaccgtcggcaaactcgtcaagcttggctacgacgtcgccgtgcaggctgacgccggcctggctgcaaagttcaccgacgcggactacgaatccgcaggtgccgccattgtcgacgagtctgtctggcacagcgatatcgtcgtaacgctcgacactccgccggagcagttccgcgcactgcttaacgacggcgccatgctggtcagccgacttgcgccaggccgtaacgaagagctggtcgaagagctcgcgcaccgcaacatcactgcccttgctatggacgcagttccccgcatctcccgggcacagtcgatggacgtgctgtcgtcgatggccaacatcggcggctaccgcgcagtagtcgaagcggcttctgcatatggtcgccttttcactggtcaggtgactgccgcaggcaagatgccgccagctaccgtttacgtcatcggcgctggtgtcggcggacttgccgcaatcggtaccgccaactctatgggcgcgattgtcaaggcaacagacctgcgccctgaagccggtgaacaggtcgaatcgatgggtgcagagttcatcccgattccggccgccactgagaagtccgaagatggctacgccaaggaaatgaccaatgatcaggctgccgctgccgcgaagctctactccgagcagtccgcgcaagctgacattgtcatcaccaccgcgaatatcccgggccgtcgctctccgctgctgctgactgctgccgatgttgcagctatgaaaccaggcagcgtcatcgtcgacatggctgccgccggtggcggtaactgcgagatgacagttccaggcaagaccattgtcactgacaacggtgtgaccatcatcggttacaccgaccttgcagggcgtctgcctgcgcaggcatcgtcgctgtacggtcagaacattttcaacctgttcaagctgattacgccagaaaaggatggctctccagttctcaatctcgaggacgagattatccgtggcatcacggtgacaaaggctcgcccacagaatggcgccggcgctaccggagctgagattctctggccaccaccgcccatcaaggtcgctgtcacccctgctgccccgctgcaggaacagcaggctcagcaggctgcattagaagagaatgctccggagaaggtttccttcatgggatcgggcatgggctcgaagattgctctgggcctgacggcactgctggcaattgtggttatgctcagcgcaccgcacagcgtgagcgccaacttcatggttctcaccttggctatcgtgcttggcttctacgtgatctctgcggtcacgccgcgcctgcacacaccgctgatgtctgagaccaacgcgatttccggcattgttctggtgggtgcgattctccaggtgggaagctccaacctgttagtttccggtctcgcgttcgcggccatcgtagtcagctccatcaatatcttcggcggtttcgccgtcaccgaccgcatgcttggcatgttcgtgaaagaggaggcataa

SEQ ID NO: 47 - DNA, 1476 bp, Corynebacterium amycolatum
  source 1..1476: mol_type = other DNA
atggctagcattgatactgcttcgcttctggactggacctaccgcctgtccaacgtcggctacattgtcgccgccgtcctgttcctcgctgcactctcgggcctgtccaagccggagaccgctcgccgcggaaacgccttcggtattgccggcatggccgtcgccgttgtcatcgccatcttccaggcactcgttaccgctgacaccaagccggattctcacttctccccgctgattaccctgattctcatcgctgtcgctatcggcatcggtggtgtcatcggtatcagtcgcgcacgcagcgttgccatgactggtatgccgcagctgattgcactgttcaacggtctggttggactcggcgctatcttcatcggcttcaactcctacatcttcgccgaagatgtcgcccccgatgccctgaagttccacttcggcgaggtttacattggcgtcttcatcggcgccgtgactttcactggctccatcgtcgcaggcctgaagctgtctgagaagatcaagggctcgccgctactgctgccgggccgcaacgctctgaacattgccattctggtggtcactctggttctcctggctgtcttcatcgcaaccggcaccgagggcggcgccatcgcatgggcatgcatggttgcagtcactgctttgggcctgttcttgggctggcacctggtcatcgccatcggtggcggcgatatgccggttgtcgtgtccatcatgaactcgtactccgggtgggccgctgctttcaccggtctcatgcttggcaacccgctgctcatcatcactggtgcgctggttggttcctccggcgcctacctgtcgtacatcatgtgtgaggccatgaaccgctcctttgccaacgttattctgggtggctttggctccgaggcttcgtcgggaagcgccgtggaaggctcccacaccgaggtcagccacgaggacacctccgagattctgcgtgacgcagacaagattctcatcgctccgggctacggtatggctgtggcacaggctcagtacgctgttgctgacctggtccgtaatctgcgtgacgccggcaaggaagtggtcttcggtatccacccagtcgctggccgcctgccgggtcacatgaacgtgctgttggcagaggccaaggttccctacgacatcgtgctggagctggacgaggtcaacgatgatttcgctgatgtggatgtcaccctggtcatcggcgcaaatgacaccgtcaacccgatggcagagcagccgggctccccgattgcgggtatgccggtgctgaaggtgtgggaatctgagcgcgtgattgttctcaagcggtcgatgggttcgggctactcgggcgtgcagaacccgctgttcttcaacgaaaacaccgacatgcttatcggcgatgcgaaggccagcatcgactccctgaatcgcatcctggcggattcgaaggtcaacgcttaa

SEQ ID NO: 48 - DNA, 1608 bp, Cellulosimicrobium funkei
  source 1..1608: mol_type = other DNA
atgcgcatcggtgtgccccgtgaagtacgggatggtgaacggctcgtagccgctactccgcgtaccgtagaacgtcttcgcgccctgggctatgacgtcgtggtcgagcacgatgccggagcgggcgccacgttctcggatgctgcttacgaggctgcaggtgcggcggtggtggatgctgccgcggcttggggcgctgatgtcgttactgccgtgaatgcccccactgacgcacaggttgccttgctgcggcctggtgccacgctggtcgccatgctcggccctgcgaatgaccccgaccttgtacaacggcttgccgcccatggtgttaccgcattggctttggacgcggtcccacgtatttctcgcgcacaagccttggacgtcctgagcacgctctctaacgttgcgggctaccgggcggtggtcgaggcagccggcgagtacggtggaatgtttgctggacaggttactgcagcgggaaaaaccccgcccgcccgggttttcgtgattggaggcggtgttgcgggccttgcagcagttggcgctgcggcatctttgggcgcccaagtgcgcgcgttcgacgtacggtcggaggccgcggaacagatcgagtctatgggcggtacggcagtgcgtgagcctgcggcccagcagggaatgtcggcagacggctatgcgaaaccgttgaccccagagcaggaagcagccgctctggcggtgtatgctcgtgaggcagccgaagcagatgtcgtcatcacgaccgcgctcgtacgcggccgtgctccccggacgctgaccgcagaagcagtggctggcatgcgtcccggtagcgtagtggtagacttggctgcttcaggaggaggtaactgtgcgctcaccgttcccggagagcgggttgtaactgaggacggcgtggtggtagtcggctggaccgacttggcaggtcgtcttcctcagcacacctcacaacttctgggaacgaacgtagtgcatcttctcgaactcctcaccccaggtaaggacggaaccttggccctggatttggacgatcctgtgcaacgtggtatgactgtggcgcgcgatggagatgtgttgtggcctccgccccctgtcgctgtatcggcagctcctgcacccggcagcacggtgcctccgccgccacccgaccctgcccaagaagctgcagatcgcgaacgcgcagccgccgaagccgcatccgctgcctctctgcgtcgtcgccgtcgtaccgttggcgctgcactcgccgcagtccttgtcacgcttgccttgtccttcgcgccgccgtcgttggtcggccatgtcactgttttcacgctggccgttgtagtaggttactatgtaatttccaatgttacccattccttgcacacccccctcatggcccagactaacgctatttcaggaattattttggttggtgcgctgcttcaaattggatccgacgactgggtcgtcactactcttgccctgctcgctgccactgtagcctctattaacattttcggcggattcttggtggctaaccgcatgatccggatgttccggaaagacgctccagcgcgcgcacagggagttgctcggtga

SEQ ID NO: 49 - DNA, 1413 bp, Cellulosimicrobium funkei
  source 1..1413: mol_type = other DNA
atgaccgcgacctcggtagcccaggcggtctacgtccttgccgctgtcttgttcgtcctgtcactggccggactgtcaaagcaggaaagcgcacggcgcggtaaccttttgggtatggtcggaatggttcttgcacttgctgcgaccattgtactggctctcggcacgtctgcacggccagttctcgtgactgcattgctgatcgccttggttcttctggtaggtgcggctgtaggtacttggcgcgcgcgtcgtgtggaaatgactcagatgcccgagttgattgccattctgcatagctttgtgggtgctgcagctgtgcttgtgggcttcaacagctacttgaccgctcatgcggcaggtgcagatgatgttgcgcacctggtggaggtcagcctcggcgtactggtaggtgctgtgacctttacgggttctgtagtcgcatttcttaagttgtccggtcgcactcggtctgcgccactccaactcccaggtcggaatctccttaatctcgcggcattgctggttagcttgggacttgttgtatggtttgttgttgctccctccatttggccgcttctgttgctgactgttgtaagcttggcgctcggctggcaccttgtggctagcattggaggtggcgacatgccggtagtcgtgtctatgctcaacagctattccggctgggcggcagcggcagcaggatttatgctgggtaacgacctgcttattgttactggagcccttgtcggttcttccggagcaattcttagctatatcatgtgtaaggctatgaatcggtctttcgtgtcggttattctgggcggcttcggtgctgaggagggtgctgcccctgcgggaggcggagagggaccacagggcgaacaccgggaagtttcagccgacgaagttgctgcgttgttgcgggatgcccgctcggttgtcattaccccgggctacggcatggctgtggcaaaagcacagtatccggtcgcagaacttgtggaattgttgcgcgacggcggagctgaggtccggttcggagttcaccctgtggcaggccggctgccaggccacatgaatgtcctgctggcggaagcacgcgtcccatatgatattgttctcgaaatggacgagatcaatgacgaccttgctggcaccgacgtggtgctggttattggtgcgaatgacaccgtgaacccggcggctcttgatgatccgggttcgccgattgccggtatgccggtgcttcacgtatgggaagcaggccaggtagtcgttttcaaacgttccatggctgccggatacgcaggcgtccagaaccctttgttcttccgtgaaaatacgggaatgcttttcggtgacgctaaacaacgggtagaggacatcgtcgctgcgctgcgggtgggttga

SEQ ID NO: 50 - DNA, 5802 bp, synthetic construct
  source 1..5802: mol_type = other DNA
gttcgcttgctgtccataaaaccgcccagtctagctatcgccatgtaagcccactgcaagctacctgctttctctttgcgcttgcgttttcccttgtccagatagcccagtagctgacattcatccggggtcagcaccgtttctgcggactggctttctacgtgttccgcttcctttagcagcccttgcgccctgagtgcttgcggcagcgtgaagctagcttttatcgccattcgccattcaggctgcgcaactgttgggaagggcgatcggtgcgggcctcttcgctattacgccagctggcgaaagggggatgtgctgcaaggcgattaagttgggtaacgccagggttttcccagtcacgacgttgtaaaacgacggccagtgaattcgagctcggtacccggggatcctctagagtcgacctgcaggcatgcaagcttggcgtaatcatggtcatagctgtttcctgtgtgaaattgttatccgctcacaattccacacaacatacgagccggaagcataaagtgtaaagcctggggtgcctaatgagtgagctaactcacattaattgcgttgcgctcactgcccgctttccagtcgggaaacctgtcgtgccagctgcattaatgaatcggccaacgcgcggggagaggcggtttgcgtattgggcgctcttccgcttcctcgctcactgactcgctgcgctcggtcgttcggctgcggcgagcggtatcagctcactcaaaggcggtaatacggttatccacagaatcaggggataacgcaggaaagaacatgtgagcaaaaggccagcaaaaggccaggaaccgtaaaaaggccgcgttgctggcgtttttccataggctccgcccccctgacgagcatcacaaaaatcgacgctcaagtcagaggtggcgaaacccgacaggactataaagataccaggcgtttccccctggaagctccctcgtgcgctctcctgttccgaccctgccgcttaccggatacctgtccgcctttctcccttcgggaagcgtggcgctttctcaatgctcacgctgtaggtatctcagttcggtgtaggtcgttcgctccaagctgggctgtgtgcacgaaccccccgttcagcccgaccgctgcgccttatccggtaactatcgtcttgagtccaacccggtaagacacgacttatcgccactggcagcagccactggtaacaggattagcagagcgaggtatgtaggcggtgctacagagttcttgaagtggtggcctaactacggctacactagaaggacagtatttggtatctgcgctctgctgaagccagttaccttcggaaaaagagttggtagctcttgatccggcaaacaaaccaccgctggtagcggtggtttttttgtttgcaagcagcagattacgcgcagaaaaaaaggatctcaagaagatcctttgatcttttctacggggtctgacgctcagtggaacgaaaactcacgttaagggattttggtcatgagattatcaaaaaggatcttcacctagatccttttggggtgggcgaagaactccagcatgagatccccgcgctggaggatcatccagccctgatagaaacagaagccactggagcacctcaaaaacaccatcatacactaaatcagtaagttggcagcatcacccgacgcactttgcgccgaataaatacctgtgacggaagatcacttcgcagaataaataaatcctggtgtccctgttgataccgggaagccctgggccaacttttggcgaaaatgagacgttgatcggcacgtaagaggttccaactttcaccataatgaaataagatcactaccgggcgtattttttgagttatcgagattttcaggagctgatagaaacagaagccactggagcacctcaaaaacaccatcatacactaaatcagtaagttggcagcatcacccgacgcactttgcgccgaataaatacctgtgacggaagatcacttcgcagaataaataaatcctggtgtccctgttgataccgggaagccctgggccaacttttggcgaaaatgagacgttgatcggcacgtaagaggttccaactttcaccataatgaaataagatcactaccgggcgtattttttgagttatcgagattttcaggagctctttggcatcgtctctcgcctgtcccctcagttcagtaatttcctgcatttgcctgtttccagtcggtagatattccacaaaacagcagggaagcagcgcttttccgctgcataaccctgcttcggggtcattatagcgattttttcggtatatccatcctttttcgcacgatatacaggattttgccaaagggttcgtgtagactttccttggtgtatccaacggcgtcagccgggcaggataggtgaagtaggcccacccgcgagcgggtgttccttcttcactgtcccttattcgcacctggcggtgctcaacgggaatcctgctctgcgaggctggccggctaccgccggcgtaacagatgagggcaagcggatggctgatgaaaccaagccaaccaggaagggcagcccacctatcaaggtgtactgccttccagacgaacgaagagcgattgaggaaaaggcggcggcggccggcatgagcctgtcggcctacctgctggccgtcggccagggctacaaaatcacgggcgtcgtggactatgagcacgtccgcgagggcgtcccggaaaacgattccgaagcccaacctttcatagaaggcggcggtggaatcgaaatctcgtgatggcaggttgggcgtcgcttggtcggtcatttcgaaaaaggttaggaatacggttagccatttgcctgcttttatatagttcatatgggattcacctttatgttgataagaaataaaagaaaatgccaataggatatcggcattttcttttgcgtttttatttgttaactgttaattgtccttgttcaaggatgctgtctttgacaacagatgttttcttgcctttgatgttcagcaggaagctcggcgcaaacgttgattgtttgtctgcgtagaatcctctgtttgtcatatagcttgtaatcacgacattgtttcctttcgcttgaggtacagcgaagtgtgagtaagtaaaggttacatcgttaggcggatcaagatccatttttaacacaaggccagttttgttcagcggcttgtatgggccagttaaagaattagaaacataaccaagcatgtaaatatcgttagacgtaatgccgtcaatcgtcatttttgatccgcgggagtcagtgaacaggtaccatttgccgttcattttaaagacgttcgcgcgttcaatttcatctgttactgtgttagatgcaatcagcggtttcatcacttttttcagtgtgtaatcatcgtttagctcaatcataccgagagcgccgtttgctaactcagccgtgcgttttttatcgctttgcagaagtttttgactttcttgacggaagaatgatgtgcttttgccatagtatgctttgttaaataaagattcttcgccttggtagccatcttcagttccagtgtttgcttcaaatactaagtatttgtggcctttatcttctacgtagtgaggatctctcagcgtatggttgtcgcctgagctgtagttgccttcatcgatgaactgctgtacattttgatacgtttttccgtcaccgtcaaagattgatttataatcctctacaccgttgatgttcaaagagctgtctgatgctgatacgttaacttgtgcagttgtcagtgtttgtttgccgtaatgtttaccggagaaatcagtgtagaataaacggatttttccgtcagatgtaaatgtggctgaacctgaccattcttgtgtttggtcttttaggatagaatcatttgcatcgaatttgtcgctgtctttaaagacgcggccagcgtttttccagctgtcaatagaagtttcgccgactttttgatagaacatgtaaatcgatgtgtcatccgcatttttaggatctccggctaatgcaaagacgatgtggtagccgtgatagtttgcgacagtgccgtcagcgttttgtaatggccagctgtcccaaacgtccaggccttttgcagaagagatatttttaattgtggacgaatcaaattcagaaacttgatatttttcatttttttgctgttcagggatttgcagcatatcatggcgtgtaatatgggaaatgccgtatgtttccttatatggcttttggttcgtttctttcgcaaacgcttgagttgcgcctcctgccagcagtgcggtagtaaaggttaatactgttgcttgttttgcaaactttttgatgttcatcgttcatgtctccttttttatgtactgtgttagcggtctgcttcttccagccctcctgtttgaagatggcaagttagttacgcacaataaaaaaagacctaaaatatgtaaggggtgacgccaaagtatacactttgccctttacacattttaggtcttgcctgctttatcagtaacaaacccgcgcgatttacttttcgacctcattctattagactctcgtttggattgcaactggtctattttcctcttttgtttgatagaaaatcataaaaggatttgcagactacgggcctaaagaactaaaaaatctatctgtttcttttcattctctgtattttttatagtttctgttgcatgggcataaagttgcctttttaatcacaattcagaaaatatcataatatctcatttcactaaataatagtgaacggcaggtatatgtgatgggttaaaaaggatcaccccagagtcccgctcagaagaactcgtcaagaaggcgatagaaggcgatgcgctgcgaatcgggagcggcgataccgtaaagcacgaggaagcggtcagcccattcgccgccaagctcttcagcaatatcacgggtagccaacgctatgtcctgatagcggtccgccacacccagccggccacagtcgatgaatccagaaaagcggccattttccaccatgatattcggcaagcaggcatcgccatgggtcacgacgagatcctcgccgtcgggcatccgcgccttgagcctggcgaacagttcggctggcgcgagcccctgatgctcttcgtccagatcatcctgatcgacaagaccggcttccatccgagtacgtgctcgctcgatgcgatgtttcgcttggtggtcgaatgggcaggtagccggatcaagcgtatgcagccgccgcattgcatcagccatgatggatactttctcggcaggagcaaggtgagatgacaggagatcctgccccggcacttcgcccaatagcagccagtcccttcccgcttcagtgacaacgtcgagacagctgcgcaaggaacgcccgtcgtggccagccacgatagccgcgctgcctcgtcttggagttcattcagggcaccggacaggtcggtcttgacaaaaagaaccgggcgcccctgcgctgacagccggaacacggcggcatcagagcagccgattgtctgttgtgcccagtcatagccgaatagcctctccacccaagcggccggagaacctgcgtgcaatccatcttgttcaatcatgcgaaacgatcctcatcctgtctcttgatcagatcttgatcccctgcgccatcagatccttggcggcaagaaagccatccagtttactttgcagggcttcccaaccttaccagagggcgccccagctggcaattccg